European Patent Application EP 4 600 337 A2, published August 13, 2025. Title: Bacillus gibsonii Protease und Varianten davon. Applicant: Henkel AG & Co. KGaA. The sequence listing filed with the application follows.

SEQUENCE LISTING (9 sequences)

SEQ ID NO: 1 - protein, 269 aa, Bacillus gibsonii
QQTVPWGITRVQAPTVHNRGITGSGVKVAILDTGIAQHSDLTIRGGASFVPGESTTADLNGHGTHVAGTVAALNNSIGVIGVAPSADLYAVKVLGANGRGSVSGIAQGLEWAATNNMHIANMSLGSDAPSTTLERAVNYATSRGVLVIAATGNNGTGSIGYPARYANAMAVGATDQNNRRASFSQYGTGIDIVAPGVGIQSTYLNNSYASMPGTSMATPHVAGVAALVKQKNPSWNATQIRNHLKNTATNLGNSSQFGSGLVNADAATR

SEQ ID NO: 2 - protein, 269 aa, synthetic construct
  REGION 1..269: note = Protease Variante
QQTVPWGITRVQAPTVHNRGITGSGVKVAILDTGIAQHSDLTVRGGASFVPGESTTADLNGHGTHVAGTVAALNNSIGVIGVAPSADLYAVKVLGANGRGSVSGIAQGLEWAATNNMHIANMSLGSDAPSTTLERAVNYATSRGVLVIAATGNNGTGSIGYPARYANAMAVGATDQNNRRASFSQYGTGIDIVAPGVGIQSTYLNNSYASMPGTSMATPHVAGVAALVKQKNPSWNATQIRNHLKNTATNLGNSSQFGSGLVNADAATR

SEQ ID NO: 3 - protein, 269 aa, synthetic construct
  REGION 1..269: note = Protease Variante
QQTVPWGITRVQAPTVHNRGITGSGVKVAILDTGIAQHSDLTIRGGASFVPGESTTADLNGHGTHVAGTVAALNNSIGVIGVAPSADLYAVKVLGANGRGSVSGIAQGLEWAATNNMHIANLSLGSDAPSTTLERAVNYATSRGVLVIAATGNSGAGSIGYPARYANAMAVGATDQNNRRASFSQYGTGIDIVAPGVGIQSTYLNNSYASMPGTSMATPHVAGVAALVKQKNPSWNATQIRNHLKNTATNLGNSSQFGSGLVNADAATR

SEQ ID NO: 4 - protein, 269 aa, synthetic construct
  REGION 1..269: note = Protease Variante
QQTVPWGITRVQAPTVHNRGITGSGVKVAILDTGIAQHSDLTIRGGASFVPGESTTADLNGHGTHVAGTVAALNNSIGVIGVAPSADLYAVKVLGANGRGSVSGIAQGLEWAATNNMHIANMSLGSDAPSTTLERAVNYATSRGVLVIAATGNNGTGSIGYPARYANAMAVGATDQNNRRASFSQYGTGIDIVAPGVGIQSTYLNNSYASNDGTSMATPHVAGVAALVKQKNPSWNATQIRNHLKNTATNLGNSSQFGSGLVNADAATR

SEQ ID NO: 5 - protein, 269 aa, synthetic construct
  REGION 1..269: note = Protease Variante
QQTVPWGITRVQAPTVHNRGITGSGVKVAILDTGIAQHSDLTIRGGASFVPGESTTADLNGHGTHVAGTVAALNNSIGVIGVAPSADLYAVKVLGANGRGSVSGIAQGLEWAATNNMHIANMSLGSDAPSTTLERAVNYATSRGVLVIAATGNNGTGSIGYPARYANAMAVGATDQNNRRASFSQYGTGIDIVAPGVGIQSTYLNNSYASLDGTSMATPHVAGVAALVKQKNPSWNATQIRNHLKNTATNLGNSSQFGSGLVNADAATR

SEQ ID NO: 6 - protein, 269 aa, synthetic construct
  REGION 1..269: note = Protease Variante
QQTVPWGITRVQAPTVHNRGITGSGVKVAILDTGIAQHSDLTIRGGASFVPGESTTADLNGHGTHVAGTVAALNNSIGVIGVAPSADLYAVKVLGANGRGSVSGIAQGLEWAATNNMHIANMSLGSDAPSTTLERAVNYATSRGVLVIAATGNNGTGSISYPARYANAMAVGATDQNNRRASFSQYGTGIDIVAPGVGIQSTYLNNSYASMPGTSMATPHVAGVAALVKQKNPSWNATQIRNHLKNTATNLGNSSQFGSGLVNADAATR

SEQ ID NO: 7 - protein, 269 aa, synthetic construct
  REGION 1..269: note = Protease Variante
QQTVPWGITRVQAPTVHNRGITGSGVKVAILDTGIAQHSDLTIRGGASFVPGESTTADLNGHGTHVAGTVAALNNSIGVIGVAPSADLYAVKVLGANGRGSVSGIAQGLEWAATNNMHIANMSLGSPAPSTTLERAVNYATSRGVLVIAATGNNGTGSIGYPARYANAMAVGATDQNNRRASFSQYGTGIDIVAPGVGIQSTYLNNSYASLDGTSMATPHVAGVAALVKQKNPSWNATQIRNHLKNTATNLGNSSQFGSGLVNADAATR

SEQ ID NO: 8 - protein, 269 aa, synthetic construct
  REGION 1..269: note = Protease Variante
QQTVPWGITRVQAPTVHNRGITGSGVKVAILDTGIAQHSDLTIRGGASFVPGESTTADLNGHGTHVAGTVAALNNSIGVIGVAPSADLYAVKVLGANGRGSVSGIAQGLEWAATNNMHIANMSLGSDAPSTTLERAVNYATSRGVLVIAATGNNGTGSIGYPARYANAMAVGATDQNNRRASFSQYGTGIDIVAPGVGIQSTYLNNSYASMHGTSMATPHVAGVAALVKQKNPSWNATQIRNHLKNTATNLGNSSQFGSGLVNADAATR

SEQ ID NO: 9 - protein, 269 aa, synthetic construct
  REGION 1..269: note = Protease Variante
QQTVPWGITRVLAPTVHNRGITGSGVKVAILDTGIAQHSDLTIRGGASFVPGESTTADLNGHGTHVAGTVAALNNSIGVIGVAPSADLYAVKVLGANGRGSVSGIAQGLEWAATNNMHIANLSLGSDAPSTTLERAVNYATSRGVLVIAATGNNGTGSIGYPARYANAMAVGATDQNNRRASFSQYGTGIDIVAPGVGIQSTYLNNSYASMPGTSMATPHVSGVAALVKQKNPSWNATQIRNHLKNTATNLGNSSQFGSGLVNADAATR